European Patent Application EP 4 696 711 A1, published February 18, 2026. Title: ANTIGEN BINDING MOLECULE SPECIFICALLY BINDING TO EGFR AND MUC1, DRUG CONJUGATE THEREOF, AND MEDICAL USE THEREOF. Applicant: JIANGSU HENGRUI PHARMACEUTICALS CO., LTD. Application WO. The sequence listing filed with the application follows.

SEQUENCE LISTING (186 sequences)

SEQ ID NO: 1 - protein, 198 aa, synthetic construct
  CHAIN 1..198: note = MUC1-C-L-6xHis
ASGSASGSASTLVHNGTSARATTTPASKSTPFSIPSHHSDTPTTLASHSTKTDASSTHHSSVPPLTSSNHSTSPQLSTGVSFFFLSFHISNLQFNSSLEDPSTDYYQELQRDISEMFLQIYKQGGFLGLSNIKFRPGSVVVQLTLAFREGTINVHDVETQFNQYKTEAASRYNLTISDVSVSDVPFPFSAQSHHHHHH

SEQ ID NO: 2 - protein, 419 aa, synthetic construct
  CHAIN 1..419: note = hMUC1-C-L-Fc
ASGSASGSASTLVHNGTSARATTTPASKSTPFSIPSHHSDTPTTLASHSTKTDASSTHHSSVPPLTSSNHSTSPQLSTGVSFFFLSFHISNLQFNSSLEDPSTDYYQELQRDISEMFLQIYKQGGFLGLSNIKFRPGSVVVQLTLAFREGTINVHDVETQFNQYKTEAASRYNLTISDVSVSDVPFPFSAQSDKTHTCPPCPAPELLGGPSVFLFPPKPKDTLMISRTPEVTCVVVDVSHEDPEVKFNWYVDGVEVHNAKTKPREEQYNSTYRVVSVLTVLHQDWLNGKEYKCKVSNKALPAPIEKTISKAKGQPREPQVYTLPPSRDELTKNQVSLTCLVKGFYPSDIAVEWESNGQPENNYKTTPPVLDSDGSFFLYSKLTVDKSRWQQGNVFSCSVMHEALHNHYTQKSLSLSPGK

SEQ ID NO: 3 - protein, 347 aa, synthetic construct
  CHAIN 1..347: note = Cyno MUC1-C-Fc
LSLGVSFFFLSFHISNLQFNSSLEDPSTNYYQQLQRDISELFLQIYKQGDFLGLSNIMFRPGSVVVQSTLVFREGTTNVHDVETQFNQRKTEAASRYNLTISDISVRDVPFPFSAQTGAGDKTHTCPPCPAPELLGGPSVFLFPPKPKDTLMISRTPEVTCVVVDVSHEDPEVKFNWYVDGVEVHNAKTKPREEQYNSTYRVVSVLTVLHQDWLNGKEYKCKVSNKALPAPIEKTISKAKGQPREPQVYTLPPSRDELTKNQVSLTCLVKGFYPSDIAVEWESNGQPENNYKTTPPVLDSDGSFFLYSKLTVDKSRWQQGNVFSCSVMHEALHNHYTQKSLSLSPGK

SEQ ID NO: 4 - protein, 121 aa, Mus musculus
  REGION 1..121: note = M4 mVH
QVQLQQSGAELARPGASVKLSCKASGYSFTTYGVPWVKQRTGQGLEWIGDIYPRSGNTYYNEKFKGKATLTADKSSDTVFMELRSLSSEDSAVYFCAREDYDNYPYALDYWGQGTSVTVSS

SEQ ID NO: 5 - protein, 106 aa, Mus musculus
  REGION 1..106: note = M4 mVL
EIVLTQSPAIIAASPGEKVTITCSASSSVFNMNWYQQKPGSSPKIWIYDISKLASGVPGRFSGSGSGTSFSLTINSMEAEDVGTYYCQQRSFYPPTFGGGTKVEIK

SEQ ID NO: 6 - protein, 123 aa, Mus musculus
  REGION 1..123: note = M6 mVH
QVQLQQSGAELMKPGASVKLSCKATGYRFIPYWIEWIKERPGHGLEWIGEILPGTGRTNYNEKFKGKATFTADTSSNTAYMQLSSLTTEDSAIYYCARYGDDTSGGYYAVDYWGQGTSVTVSS

SEQ ID NO: 7 - protein, 111 aa, Mus musculus
  REGION 1..111: note = M6 mVL
DIVMTQSSASLAMSLGQRATISCRASESVNILGTNLIHWYQQKPGQPPKLLIYHASNLETGVPARFSGSGSRTDFTLTIDPVEEDDVAIYYCLQSRKIPWTFGGGTKLEIK

SEQ ID NO: 8 - protein, 122 aa, Mus musculus
  REGION 1..122: note = F4-1 mVH
QIQLQQSGPELVKPGASVKISCKASGYTFTDNYINWVKQRPGQGLEYIGWIYPGSGNNKFNEKFKGKATLTVDTSSRTAFMQLSSLTFEDSAVYFCARDYPFPSYHYGMDYWGQGTSVTVSS

SEQ ID NO: 9 - protein, 106 aa, Mus musculus
  REGION 1..106: note = F4-1 mVL
QILLTQSPAIMSASPGERVTITCSASSSVSYIHWFQQKPGTSPKLWIYSTSNLASGVPPRFSGSGSGTSFSLTVSRMEAEDAATYYCQQRSSYPPTFGGGTKLEIK

SEQ ID NO: 10 - protein, 117 aa, Mus musculus
  REGION 1..117: note = F4-18 mVH
EVQLQQSGAELVRPGSSVKMSCKTSGYTFTSYGINWVKQRPGQGLEWIGYIYLGSDYTEYNEKFKGKATLTSDTTSSTAYMQLSSLTSEDSAIYFCARSAGSLFAYWGQGTLVTVSA

SEQ ID NO: 11 - protein, 107 aa, Mus musculus
  REGION 1..107: note = F4-18 mVL
DIQLTQSPSSLSASLGERVSLTCRASQDIGITLNWLQQEPDGTIKRLIYATSSLDSGVPKRFSGSRSGSDYSLTISSLESEDFVDYYCLQYASSPYTFGGGTKLEIK

SEQ ID NO: 12 - protein, 5 aa, Mus musculus
  REGION 1..5: note = M4-HCDR1
TYGVP

SEQ ID NO: 13 - protein, 17 aa, Mus musculus
  REGION 1..17: note = M4-HCDR2
DIYPRSGNTYYNEKFKG

SEQ ID NO: 14 - protein, 12 aa, Mus musculus
  REGION 1..12: note = M4-HCDR3
EDYDNYPYALDY

SEQ ID NO: 15 - protein, 10 aa, Mus musculus
  REGION 1..10: note = M4-LCDR1
SASSSVFNMN

SEQ ID NO: 16 - protein, 7 aa, Mus musculus
  REGION 1..7: note = M4-LCDR2
DISKLAS

SEQ ID NO: 17 - protein, 9 aa, Mus musculus
  REGION 1..9: note = M4-LCDR3
QQRSFYPPT

SEQ ID NO: 18 - protein, 5 aa, Mus musculus
  REGION 1..5: note = M6-HCDR1
PYWIE

SEQ ID NO: 19 - protein, 17 aa, Mus musculus
  REGION 1..17: note = M6-HCDR2
EILPGTGRTNYNEKFKG

SEQ ID NO: 20 - protein, 14 aa, Mus musculus
  REGION 1..14: note = M6-HCDR3
YGDDTSGGYYAVDY

SEQ ID NO: 21 - protein, 15 aa, Mus musculus
  REGION 1..15: note = M6-LCDR1
RASESVNILGTNLIH

SEQ ID NO: 22 - protein, 7 aa, Mus musculus
  REGION 1..7: note = M6-LCDR2
HASNLET

SEQ ID NO: 23 - protein, 9 aa, Mus musculus
  REGION 1..9: note = M6-LCDR3
LQSRKIPWT

SEQ ID NO: 24 - protein, 5 aa, Mus musculus
  REGION 1..5: note = F4-1-HCDR1
DNYIN

SEQ ID NO: 25 - protein, 17 aa, Mus musculus
  REGION 1..17: note = F4-1 HCDR2
WIYPGSGNNKFNEKFKG

SEQ ID NO: 26 - protein, 13 aa, Mus musculus
  REGION 1..13: note = F4-1-HCDR3
DYPFPSYHYGMDY

SEQ ID NO: 27 - protein, 10 aa, Mus musculus
  REGION 1..10: note = F4-1-LCDR1
SASSSVSYIH

SEQ ID NO: 28 - protein, 7 aa, Mus musculus
  REGION 1..7: note = F4-1-LCDR2
STSNLAS

SEQ ID NO: 29 - protein, 9 aa, Mus musculus
  REGION 1..9: note = F4-1-LCDR3
QQRSSYPPT

SEQ ID NO: 30 - protein, 5 aa, Mus musculus
  REGION 1..5: note = F4-18-HCDR1
SYGIN

SEQ ID NO: 31 - protein, 17 aa, Mus musculus
  REGION 1..17: note = F4-18-HCDR2
YIYLGSDYTEYNEKFKG

SEQ ID NO: 32 - protein, 8 aa, Mus musculus
  REGION 1..8: note = F4-18-HCDR3
SAGSLFAY

SEQ ID NO: 33 - protein, 11 aa, Mus musculus
  REGION 1..11: note = F4-18-LCDR1
RASQDIGITLN

SEQ ID NO: 34 - protein, 7 aa, Mus musculus
  REGION 1..7: note = F4-18-LCDR2
ATSSLDS

SEQ ID NO: 35 - protein, 9 aa, Mus musculus
  REGION 1..9: note = F4-18-LCDR3
LQYASSPYT

SEQ ID NO: 36 - protein, 121 aa, synthetic construct
  REGION 1..121: note = huM4VH1
EVQLVQSGAEVKKPGASVKVSCKASGYTFTTYGVPWVRQAPGQGLEWMGDIYPRSGNTYYNEKFKGRVTMTADKSTDTVYMELSSLRSEDTAVYYCAREDYDNYPYALDYWGQGTTVTVSS

SEQ ID NO: 37 - protein, 121 aa, synthetic construct
  REGION 1..121: note = huM4VH2
EVQLVQSGAEVKKPGASVKVSCKASGYSFTTYGVPWVRQRPGQGLEWIGDIYPRSGNTYYNEKFKGRVTMTADKSTDTVYMELSSLRSEDTAVYYCAREDYDNYPYALDYWGQGTTVTVSS

SEQ ID NO: 38 - protein, 121 aa, synthetic construct
  REGION 1..121: note = huM4VH3
EVQLVQSGAEVKKPGASVKVSCKASGYSFTTYGVPWVKQRPGQGLEWIGDIYPRSGNTYYNEKFKGRVTMTADKSTDTVYMELRSLRSEDTAVYYCAREDYDNYPYALDYWGQGTTVTVSS

SEQ ID NO: 39 - protein, 106 aa, synthetic construct
  REGION 1..106: note = huM4VL1
DIQMTQSPSSLSASVGDRVTITCSASSSVFNMNWYQQKPGKSPKLWIYDISKLASGVPSRFSGSGSGTDFTLTISSLQPEDFATYYCQQRSFYPPTFGGGTKVEIK

SEQ ID NO: 40 - protein, 106 aa, synthetic construct
  REGION 1..106: note = huM4VL2
DIVMTQSPSSLSASVGDRVTITCSASSSVFNMNWYQQKPGKSPKLWIYDISKLASGVPSRFSGSGSGTDFTLTISSLQPEDFATYYCQQRSFYPPTFGGGTKVEIK

SEQ ID NO: 41 - protein, 106 aa, synthetic construct
  REGION 1..106: note = huM4VL3
EIVLTQSPDFQSVTPKEKVTITCSASSSVFNMNWYQQKPDQSPKLWIYDISKLASGVPSRFSGSGSGTDFTLTINSLEAEDAATYYCQQRSFYPPTFGGGTKVEIK

SEQ ID NO: 42 - protein, 106 aa, synthetic construct
  REGION 1..106: note = huM4VL4
EIVLTQSPATLSLSPGERATLSCSASSSVFNMNWYQQKPGQSPRLWIYDISKLASGIPGRFSGSGSGTDFTLTISSLEPEDFAVYYCQQRSFYPPTFGGGTKVEIK

SEQ ID NO: 43 - protein, 123 aa, synthetic construct
  REGION 1..123: note = huM6VH1
EVQLVQSGAEVKKPGASVKVSCKASGYTFTPYWIEWVRQAPGQGLEWMGEILPGTGRTNYNEKFKGRVTFTADTSTNTVYMELSSLRSEDTAVYYCARYGDDTSGGYYAVDYWGQGTTVTVSS

SEQ ID NO: 44 - protein, 123 aa, synthetic construct
  REGION 1..123: note = huM6VH2
EVQLVQSGAEVKKPGASVKVSCKASGYRFIPYWIEWVRQAPGQGLEWMGEILPGTGRTNYNEKFKGRVTFTADTSTNTVYMELSSLRSEDTAVYYCARYGDDTSGGYYAVDYWGQGTTVTVSS

SEQ ID NO: 45 - protein, 123 aa, synthetic construct
  REGION 1..123: note = huM6VH3
EVQLVQSGAEVKKPGASVKVSCKASGYRFIPYWIEWVRQRPGQGLEWMGEILPGTGRTNYNEKFKGRVTFTADTSTNTVYMELSSLRSEDTAVYYCARYGDDTSGGYYAVDYWGQGTTVTVSS

SEQ ID NO: 46 - protein, 123 aa, synthetic construct
  REGION 1..123: note = huM6VH4
EVQLVQSGAEVKKPGASVKVSCKASGYRFIPYWIEWVRERPGHGLEWMGEILPGTGRTNYNEKFKGRVTFTADTSTNTVYMELSSLTSEDTAVYYCARYGDDTSGGYYAVDYWGQGTTVTVSS

SEQ ID NO: 47 - protein, 123 aa, synthetic construct
  REGION 1..123: note = huM6VH5
EVQLVQSGAEVKKPGASVKVSCKASGYRFIPYWIEWVRERPGHGLEWMGEILPGTGRTNYNEKFKGRVTFTADTSTNTVYMELSSLTSEDTAVYYCARYGEDTSGGYYAVDYWGQGTTVTVSS

SEQ ID NO: 48 - protein, 123 aa, synthetic construct
  REGION 1..123: note = huM6VH6
EVQLVQSGAEVKKPGASVKVSCKASGYRFIPYWIEWVRERPGHGLEWMGEILPGTGRTNYNEKFKGRVTFTADTSTNTVYMELSQLTSEDTAVYYCARYGEDTSGGYYAVDYWGQGTTVTVSS

SEQ ID NO: 49 - protein, 123 aa, synthetic construct
  REGION 1..123: note = huM6VH7
EVQLVQSGAEVKKPGASVKVSCKASGYRFIPYWIEWVRERPGHGLEWMGEILPGTGRTNYNEKFKGRVTFTADTSTNTVYMELSSLTNEDTAVYYCARYGEDTSGGYYAVDYWGQGTTVTVSS

SEQ ID NO: 50 - protein, 111 aa, synthetic construct
  REGION 1..111: note = huM6VL1
DIVMTQSPDSLAVSLGERATINCRASESVNILGTNLIHWYQQKPGQPPKLLIYHASNLETGVPDRFSGSGSRTDFTLTISSLQAEDVAVYYCLQSRKIPWTFGGGTKVEIK

SEQ ID NO: 51 - protein, 111 aa, synthetic construct
  REGION 1..111: note = huM6VL2
EIVLTQSPATLSLSPGERATLSCRASESVNILGTNLIHWYQQKPGQAPKLLIYHASNLETGIPARFSGSGSRTDFTLTISSLEPEDFAVYYCLQSRKIPWTFGGGTKVEIK

SEQ ID NO: 52 - protein, 111 aa, synthetic construct
  REGION 1..111: note = huM6VL3
DIVMTQSPATLSLSPGERATLSCRASESVNILGTNLIHWYQQKPGQAPKLLIYHASNLETGIPARFSGSGSRTDFTLTISSLEPEDVAVYYCLQSRKIPWTFGGGTKVEIK

SEQ ID NO: 53 - protein, 122 aa, synthetic construct
  REGION 1..122: note = huF4-1VH1
EVQLVQSGAEVKKPGASVKVSCKASGYTFTDNYINWVRQAPGQRLEYMGWIYPGSGNNKFNEKFKGRVTITVDTSASTAYMELSSLRSEDTAVYYCARDYPFPSYHYGMDYWGQGTTVTVSS

SEQ ID NO: 54 - protein, 122 aa, synthetic construct
  REGION 1..122: note = huF4-1VH2
EVQLVQSGAEVKKPGASVKVSCKASGYTFTDNYINWVRQAPGQRLEYIGWIYPGSGNNKFNEKFKGRVTLTVDTSARTAYMELSSLRSEDTAVYYCARDYPFPSYHYGMDYWGQGTTVTVSS

SEQ ID NO: 55 - protein, 122 aa, synthetic construct
  REGION 1..122: note = huF4-1VH3
EIQLVQSGAEVVKPGASVKVSCKASGYTFTDNYINWVRQRPGQGLEYIGWIYPGSGNNKFNEKFKGRVTLTVDTSARTAYMELSSLRSEDTAVYYCARDYPFPSYHYGMDYWGQGTTVTVSS

SEQ ID NO: 56 - protein, 106 aa, synthetic construct
  REGION 1..106: note = huF4-1VL1
DIQMTQSPSSLSASVGDRVTITCSASSSVSYIHWFQQKPGKAPKLWIYSTSNLASGVPSRFSGSGSGTDFTLTISSLQPEDFATYYCQQRSSYPPTFGGGTKVEIK

SEQ ID NO: 57 - protein, 106 aa, synthetic construct
  REGION 1..106: note = huF4-1VL2
DIQLTQSPSSLSASVGDRVTITCSASSSVSYIHWFQQKPGKAPKLWIYSTSNLASGVPSRFSGSGSGTDFTLTVSSLQPEDFATYYCQQRSSYPPTFGGGTKVEIK

SEQ ID NO: 58 - protein, 106 aa, synthetic construct
  REGION 1..106: note = huF4-1VL3
DIQLTQSPSSLSASVGDRVTITCSASSSVSYIHWFQQKPGTSPKLWIYSTSNLASGVPSRFSGSGSGTDFTLTVSSLQPEDFATYYCQQRSSYPPTFGGGTKVEIK

SEQ ID NO: 59 - protein, 106 aa, synthetic construct
  REGION 1..106: note = huF4-1VL4
DIQLTQSPSSLSASVGDRVTITCSASSSVSYIHWFQQKPGTSPKLWIYSTSNLASGVPPRFSGSGSGTSFTLTVSSLQPEDFATYYCQQRSSYPPTFGGGTKVEIK

SEQ ID NO: 60 - protein, 117 aa, synthetic construct
  REGION 1..117: note = huF4-18VH1
EVQLVQSGAEVKKPGASVKVSCKASGYTFTSYGINWVRQAPGQRLEWMGYIYLGSDYTEYNEKFKGRVTLTSDTSASTAYMELSSLRSEDTAVYYCARSAGSLFAYWGQGTLVTVSS

SEQ ID NO: 61 - protein, 117 aa, synthetic construct
  REGION 1..117: note = huF4-18VH2
EVQLVQSGAEVKKPGASVKVSCKASGYTFTSYGINWVRQRPGQGLEWIGYIYLGSDYTEYNEKFKGRVTLTSDTSASTAYMELSSLRSEDTAVYYCARSAGSLFAYWGQGTLVTVSS

SEQ ID NO: 62 - protein, 117 aa, synthetic construct
  REGION 1..117: note = huF4-18VH3
EVQLVQSGAEVVKPGASVKMSCKTSGYTFTSYGINWVRQRPGQGLEWIGYIYLGSDYTEYNEKFKGRVTLTSDTSASTAYMELSSLRSEDTAVYYCARSAGSLFAYWGQGTLVTVSS

SEQ ID NO: 63 - protein, 117 aa, synthetic construct
  REGION 1..117: note = huF4-18VH4
EVQLVQSGAEVVKPGASVKMSCKTSGYTFTSYGINWVRQRPGQGLEWIGYIYLGSDYTEYNEKFKGRVTLTSDTSASTAYMELSSLRSEDTAVYYCARSGGSLFAYWGQGTLVTVSS

SEQ ID NO: 64 - protein, 117 aa, synthetic construct
  REGION 1..117: note = huF4-18VH5
EVQLVQSGAEVVKPGASVKMSCKTSGYTFTSYGINWVRQRPGQGLEWIGYIYLGSDYTEYNEKFKGRVTLTSDTSASTAYMELSSLRSEDTAVYYCARSAGSLFGYWGQGTLVTVSS

SEQ ID NO: 65 - protein, 107 aa, synthetic construct
  REGION 1..107: note = huF4-18VL1
DIQMTQSPSSLSASVGDRVTITCRASQDIGITLNWYQQKPGKAPKRLIYATSSLDSGVPSRFSGSRSGTDYTLTISSLQPEDFATYYCLQYASSPYTFGGGTKVEIK

SEQ ID NO: 66 - protein, 107 aa, synthetic construct
  REGION 1..107: note = huF4-18VL2
DIQMTQSPSSLSASVGDRVTITCRASQDIGITLNWLQQKPGKAPKRLIYATSSLDSGVPSRFSGSRSGTDYTLTISSLQPEDFATYYCLQYASSPYTFGGGTKVEIK

SEQ ID NO: 67 - protein, 107 aa, synthetic construct
  REGION 1..107: note = huF4-18VL3
DIQLTQSPSSLSASVGDRVTITCRASQDIGITLNWLQQKPGKAIKRLIYATSSLDSGVPSRFSGSRSGSDYTLTISSLQPEDFATYYCLQYASSPYTFGGGTKVEIK

SEQ ID NO: 68 - protein, 107 aa, synthetic construct
  REGION 1..107: note = huF4-18VL4
DIQLTQSPSSLSASVGDRVTITCRASQDIGITLNWLQQEPGGAIKRLIYATSSLDSGVPKRFSGSRSGSDYTLTISSLQPEDFATYYCLQYASSPYTFGGGTKVEIK

SEQ ID NO: 69 - protein, 330 aa, synthetic construct [sequence omitted]

SEQ ID NO: 70 - protein, 107 aa, synthetic construct [sequence omitted]

SEQ ID NO: 71 - protein, 451 aa, synthetic construct
  CHAIN 1..451: note = M4-H1L1 heavy chain
EVQLVQSGAEVKKPGASVKVSCKASGYTFTTYGVPWVRQAPGQGLEWMGDIYPRSGNTYYNEKFKGRVTMTADKSTDTVYMELSSLRSEDTAVYYCAREDYDNYPYALDYWGQGTTVTVSSASTKGPSVFPLAPSSKSTSGGTAALGCLVKDYFPEPVTVSWNSGALTSGVHTFPAVLQSSGLYSLSSVVTVPSSSLGTQTYICNVNHKPSNTKVDKKVEPKSCDKTHTCPPCPAPELLGGPSVFLFPPKPKDTLMISRTPEVTCVVVDVSHEDPEVKFNWYVDGVEVHNAKTKPREEQYNSTYRVVSVLTVLHQDWLNGKEYKCKVSNKALPAPIEKTISKAKGQPREPQVYTLPPSRDELTKNQVSLTCLVKGFYPSDIAVEWESNGQPENNYKTTPPVLDSDGSFFLYSKLTVDKSRWQQGNVFSCSVMHEALHNHYTQKSLSLSPGK

SEQ ID NO: 72 - protein, 213 aa, synthetic construct
  CHAIN 1..213: note = M4-H1L1 light chain
DIQMTQSPSSLSASVGDRVTITCSASSSVFNMNWYQQKPGKSPKLWIYDISKLASGVPSRFSGSGSGTDFTLTISSLQPEDFATYYCQQRSFYPPTFGGGTKVEIKRTVAAPSVFIFPPSDEQLKSGTASVVCLLNNFYPREAKVQWKVDNALQSGNSQESVTEQDSKDSTYSLSSTLTLSKADYEKHKVYACEVTHQGLSSPVTKSFNRGEC

SEQ ID NO: 73 - protein, 451 aa, synthetic construct
  CHAIN 1..451: note = M4-H2L1 heavy chain
EVQLVQSGAEVKKPGASVKVSCKASGYSFTTYGVPWVRQRPGQGLEWIGDIYPRSGNTYYNEKFKGRVTMTADKSTDTVYMELSSLRSEDTAVYYCAREDYDNYPYALDYWGQGTTVTVSSASTKGPSVFPLAPSSKSTSGGTAALGCLVKDYFPEPVTVSWNSGALTSGVHTFPAVLQSSGLYSLSSVVTVPSSSLGTQTYICNVNHKPSNTKVDKKVEPKSCDKTHTCPPCPAPELLGGPSVFLFPPKPKDTLMISRTPEVTCVVVDVSHEDPEVKFNWYVDGVEVHNAKTKPREEQYNSTYRVVSVLTVLHQDWLNGKEYKCKVSNKALPAPIEKTISKAKGQPREPQVYTLPPSRDELTKNQVSLTCLVKGFYPSDIAVEWESNGQPENNYKTTPPVLDSDGSFFLYSKLTVDKSRWQQGNVFSCSVMHEALHNHYTQKSLSLSPGK

SEQ ID NO: 74 - protein, 213 aa, synthetic construct; identical to SEQ ID NO: 72
  CHAIN 1..213: note = M4-H2L1 light chain

SEQ ID NO: 75 - protein, 451 aa, synthetic construct; identical to SEQ ID NO: 71
  CHAIN 1..451: note = M4-H1L2 heavy chain

SEQ ID NO: 76 - protein, 213 aa, synthetic construct
  CHAIN 1..213: note = M4-H1L2 light chain
DIVMTQSPSSLSASVGDRVTITCSASSSVFNMNWYQQKPGKSPKLWIYDISKLASGVPSRFSGSGSGTDFTLTISSLQPEDFATYYCQQRSFYPPTFGGGTKVEIKRTVAAPSVFIFPPSDEQLKSGTASVVCLLNNFYPREAKVQWKVDNALQSGNSQESVTEQDSKDSTYSLSSTLTLSKADYEKHKVYACEVTHQGLSSPVTKSFNRGEC

SEQ ID NO: 77 - protein, 451 aa, synthetic construct; identical to SEQ ID NO: 73
  CHAIN 1..451: note = M4-H2L2 heavy chain

SEQ ID NO: 78 - protein, 213 aa, synthetic construct; identical to SEQ ID NO: 76
  CHAIN 1..213: note = M4-H2L2 light chain

SEQ ID NO: 79 - protein, 453 aa, synthetic construct
  CHAIN 1..453: note = M6-H1L1 heavy chain
EVQLVQSGAEVKKPGASVKVSCKASGYTFTPYWIEWVRQAPGQGLEWMGEILPGTGRTNYNEKFKGRVTFTADTSTNTVYMELSSLRSEDTAVYYCARYGDDTSGGYYAVDYWGQGTTVTVSSASTKGPSVFPLAPSSKSTSGGTAALGCLVKDYFPEPVTVSWNSGALTSGVHTFPAVLQSSGLYSLSSVVTVPSSSLGTQTYICNVNHKPSNTKVDKKVEPKSCDKTHTCPPCPAPELLGGPSVFLFPPKPKDTLMISRTPEVTCVVVDVSHEDPEVKFNWYVDGVEVHNAKTKPREEQYNSTYRVVSVLTVLHQDWLNGKEYKCKVSNKALPAPIEKTISKAKGQPREPQVYTLPPSRDELTKNQVSLTCLVKGFYPSDIAVEWESNGQPENNYKTTPPVLDSDGSFFLYSKLTVDKSRWQQGNVFSCSVMHEALHNHYTQKSLSLSPGK

SEQ ID NO: 80 - protein, 218 aa, synthetic construct
  CHAIN 1..218: note = M6-H1L1 light chain
DIVMTQSPDSLAVSLGERATINCRASESVNILGTNLIHWYQQKPGQPPKLLIYHASNLETGVPDRFSGSGSRTDFTLTISSLQAEDVAVYYCLQSRKIPWTFGGGTKVEIKRTVAAPSVFIFPPSDEQLKSGTASVVCLLNNFYPREAKVQWKVDNALQSGNSQESVTEQDSKDSTYSLSSTLTLSKADYEKHKVYACEVTHQGLSSPVTKSFNRGEC

SEQ ID NO: 81 - protein, 453 aa, synthetic construct
  CHAIN 1..453: note = M6-H3L1 heavy chain
EVQLVQSGAEVKKPGASVKVSCKASGYRFIPYWIEWVRQRPGQGLEWMGEILPGTGRTNYNEKFKGRVTFTADTSTNTVYMELSSLRSEDTAVYYCARYGDDTSGGYYAVDYWGQGTTVTVSSASTKGPSVFPLAPSSKSTSGGTAALGCLVKDYFPEPVTVSWNSGALTSGVHTFPAVLQSSGLYSLSSVVTVPSSSLGTQTYICNVNHKPSNTKVDKKVEPKSCDKTHTCPPCPAPELLGGPSVFLFPPKPKDTLMISRTPEVTCVVVDVSHEDPEVKFNWYVDGVEVHNAKTKPREEQYNSTYRVVSVLTVLHQDWLNGKEYKCKVSNKALPAPIEKTISKAKGQPREPQVYTLPPSRDELTKNQVSLTCLVKGFYPSDIAVEWESNGQPENNYKTTPPVLDSDGSFFLYSKLTVDKSRWQQGNVFSCSVMHEALHNHYTQKSLSLSPGK

SEQ ID NO: 82 - protein, 218 aa, synthetic construct; identical to SEQ ID NO: 80
  CHAIN 1..218: note = M6-H3L1 light chain

SEQ ID NO: 83 - protein, 453 aa, synthetic construct
  CHAIN 1..453: note = M6-H2L2 heavy chain
EVQLVQSGAEVKKPGASVKVSCKASGYRFIPYWIEWVRQAPGQGLEWMGEILPGTGRTNYNEKFKGRVTFTADTSTNTVYMELSSLRSEDTAVYYCARYGDDTSGGYYAVDYWGQGTTVTVSSASTKGPSVFPLAPSSKSTSGGTAALGCLVKDYFPEPVTVSWNSGALTSGVHTFPAVLQSSGLYSLSSVVTVPSSSLGTQTYICNVNHKPSNTKVDKKVEPKSCDKTHTCPPCPAPELLGGPSVFLFPPKPKDTLMISRTPEVTCVVVDVSHEDPEVKFNWYVDGVEVHNAKTKPREEQYNSTYRVVSVLTVLHQDWLNGKEYKCKVSNKALPAPIEKTISKAKGQPREPQVYTLPPSRDELTKNQVSLTCLVKGFYPSDIAVEWESNGQPENNYKTTPPVLDSDGSFFLYSKLTVDKSRWQQGNVFSCSVMHEALHNHYTQKSLSLSPGK

SEQ ID NO: 84 - protein, 218 aa, synthetic construct
  CHAIN 1..218: note = M6-H2L2 light chain
EIVLTQSPATLSLSPGERATLSCRASESVNILGTNLIHWYQQKPGQAPKLLIYHASNLETGIPARFSGSGSRTDFTLTISSLEPEDFAVYYCLQSRKIPWTFGGGTKVEIKRTVAAPSVFIFPPSDEQLKSGTASVVCLLNNFYPREAKVQWKVDNALQSGNSQESVTEQDSKDSTYSLSSTLTLSKADYEKHKVYACEVTHQGLSSPVTKSFNRGEC

SEQ ID NO: 85 - protein, 453 aa, synthetic construct; identical to SEQ ID NO: 81
  CHAIN 1..453: note = M6-H3L2 heavy chain

SEQ ID NO: 86 - protein, 218 aa, synthetic construct; identical to SEQ ID NO: 84
  CHAIN 1..218: note = M6-H3L2 light chain

SEQ ID NO: 87 - protein, 453 aa, synthetic construct
  CHAIN 1..453: note = M6-H4L2 heavy chain
EVQLVQSGAEVKKPGASVKVSCKASGYRFIPYWIEWVRERPGHGLEWMGEILPGTGRTNYNEKFKGRVTFTADTSTNTVYMELSSLTSEDTAVYYCARYGDDTSGGYYAVDYWGQGTTVTVSSASTKGPSVFPLAPSSKSTSGGTAALGCLVKDYFPEPVTVSWNSGALTSGVHTFPAVLQSSGLYSLSSVVTVPSSSLGTQTYICNVNHKPSNTKVDKKVEPKSCDKTHTCPPCPAPELLGGPSVFLFPPKPKDTLMISRTPEVTCVVVDVSHEDPEVKFNWYVDGVEVHNAKTKPREEQYNSTYRVVSVLTVLHQDWLNGKEYKCKVSNKALPAPIEKTISKAKGQPREPQVYTLPPSRDELTKNQVSLTCLVKGFYPSDIAVEWESNGQPENNYKTTPPVLDSDGSFFLYSKLTVDKSRWQQGNVFSCSVMHEALHNHYTQKSLSLSPGK

SEQ ID NO: 88 - protein, 218 aa, synthetic construct; identical to SEQ ID NO: 84
  CHAIN 1..218: note = M6-H4L2 light chain

SEQ ID NO: 89 - protein, 452 aa, synthetic construct
  CHAIN 1..452: note = F4-1-H1L1 heavy chain
EVQLVQSGAEVKKPGASVKVSCKASGYTFTDNYINWVRQAPGQRLEYMGWIYPGSGNNKFNEKFKGRVTITVDTSASTAYMELSSLRSEDTAVYYCARDYPFPSYHYGMDYWGQGTTVTVSSASTKGPSVFPLAPSSKSTSGGTAALGCLVKDYFPEPVTVSWNSGALTSGVHTFPAVLQSSGLYSLSSVVTVPSSSLGTQTYICNVNHKPSNTKVDKKVEPKSCDKTHTCPPCPAPELLGGPSVFLFPPKPKDTLMISRTPEVTCVVVDVSHEDPEVKFNWYVDGVEVHNAKTKPREEQYNSTYRVVSVLTVLHQDWLNGKEYKCKVSNKALPAPIEKTISKAKGQPREPQVYTLPPSRDELTKNQVSLTCLVKGFYPSDIAVEWESNGQPENNYKTTPPVLDSDGSFFLYSKLTVDKSRWQQGNVFSCSVMHEALHNHYTQKSLSLSPGK

SEQ ID NO: 90 - protein, 213 aa, synthetic construct
  CHAIN 1..213: note = F4-1-H1L1 light chain
DIQMTQSPSSLSASVGDRVTITCSASSSVSYIHWFQQKPGKAPKLWIYSTSNLASGVPSRFSGSGSGTDFTLTISSLQPEDFATYYCQQRSSYPPTFGGGTKVEIKRTVAAPSVFIFPPSDEQLKSGTASVVCLLNNFYPREAKVQWKVDNALQSGNSQESVTEQDSKDSTYSLSSTLTLSKADYEKHKVYACEVTHQGLSSPVTKSFNRGEC

SEQ ID NO: 91 - protein, 452 aa, synthetic construct; identical to SEQ ID NO: 89
  CHAIN 1..452: note = F4-1-H1L2 heavy chain

SEQ ID NO: 92 - protein, 213 aa, synthetic construct
  CHAIN 1..213: note = F4-1-H1L2 light chain
DIQLTQSPSSLSASVGDRVTITCSASSSVSYIHWFQQKPGKAPKLWIYSTSNLASGVPSRFSGSGSGTDFTLTVSSLQPEDFATYYCQQRSSYPPTFGGGTKVEIKRTVAAPSVFIFPPSDEQLKSGTASVVCLLNNFYPREAKVQWKVDNALQSGNSQESVTEQDSKDSTYSLSSTLTLSKADYEKHKVYACEVTHQGLSSPVTKSFNRGEC

SEQ ID NO: 93 - protein, 452 aa, synthetic construct
  CHAIN 1..452: note = F4-1-H2L2 heavy chain
EVQLVQSGAEVKKPGASVKVSCKASGYTFTDNYINWVRQAPGQRLEYIGWIYPGSGNNKFNEKFKGRVTLTVDTSARTAYMELSSLRSEDTAVYYCARDYPFPSYHYGMDYWGQGTTVTVSSASTKGPSVFPLAPSSKSTSGGTAALGCLVKDYFPEPVTVSWNSGALTSGVHTFPAVLQSSGLYSLSSVVTVPSSSLGTQTYICNVNHKPSNTKVDKKVEPKSCDKTHTCPPCPAPELLGGPSVFLFPPKPKDTLMISRTPEVTCVVVDVSHEDPEVKFNWYVDGVEVHNAKTKPREEQYNSTYRVVSVLTVLHQDWLNGKEYKCKVSNKALPAPIEKTISKAKGQPREPQVYTLPPSRDELTKNQVSLTCLVKGFYPSDIAVEWESNGQPENNYKTTPPVLDSDGSFFLYSKLTVDKSRWQQGNVFSCSVMHEALHNHYTQKSLSLSPGK

SEQ ID NO: 94 - protein, 213 aa, synthetic construct; identical to SEQ ID NO: 92
  CHAIN 1..213: note = F4-1-H2L2 light chain

SEQ ID NO: 95 - protein, 452 aa, synthetic construct; identical to SEQ ID NO: 89
  CHAIN 1..452: note = F4-1-H1L4 heavy chain

SEQ ID NO: 96 - protein, 213 aa, synthetic construct
  CHAIN 1..213: note = F4-1-H1L4 light chain
DIQLTQSPSSLSASVGDRVTITCSASSSVSYIHWFQQKPGTSPKLWIYSTSNLASGVPPRFSGSGSGTSFTLTVSSLQPEDFATYYCQQRSSYPPTFGGGTKVEIKRTVAAPSVFIFPPSDEQLKSGTASVVCLLNNFYPREAKVQWKVDNALQSGNSQESVTEQDSKDSTYSLSSTLTLSKADYEKHKVYACEVTHQGLSSPVTKSFNRGEC

SEQ ID NO: 97 - protein, 447 aa, synthetic construct
  CHAIN 1..447: note = F4-18-H1L1 heavy chain
EVQLVQSGAEVKKPGASVKVSCKASGYTFTSYGINWVRQAPGQRLEWMGYIYLGSDYTEYNEKFKGRVTLTSDTSASTAYMELSSLRSEDTAVYYCARSAGSLFAYWGQGTLVTVSSASTKGPSVFPLAPSSKSTSGGTAALGCLVKDYFPEPVTVSWNSGALTSGVHTFPAVLQSSGLYSLSSVVTVPSSSLGTQTYICNVNHKPSNTKVDKKVEPKSCDKTHTCPPCPAPELLGGPSVFLFPPKPKDTLMISRTPEVTCVVVDVSHEDPEVKFNWYVDGVEVHNAKTKPREEQYNSTYRVVSVLTVLHQDWLNGKEYKCKVSNKALPAPIEKTISKAKGQPREPQVYTLPPSRDELTKNQVSLTCLVKGFYPSDIAVEWESNGQPENNYKTTPPVLDSDGSFFLYSKLTVDKSRWQQGNVFSCSVMHEALHNHYTQKSLSLSPGK

SEQ ID NO: 98 - protein, 214 aa, synthetic construct
  CHAIN 1..214: note = F4-18-H1L1 light chain
DIQMTQSPSSLSASVGDRVTITCRASQDIGITLNWYQQKPGKAPKRLIYATSSLDSGVPSRFSGSRSGTDYTLTISSLQPEDFATYYCLQYASSPYTFGGGTKVEIKRTVAAPSVFIFPPSDEQLKSGTASVVCLLNNFYPREAKVQWKVDNALQSGNSQESVTEQDSKDSTYSLSSTLTLSKADYEKHKVYACEVTHQGLSSPVTKSFNRGEC

SEQ ID NO: 99 - protein, 447 aa, synthetic construct
  CHAIN 1..447: note = F4-18-H2L1 heavy chain
EVQLVQSGAEVKKPGASVKVSCKASGYTFTSYGINWVRQRPGQGLEWIGYIYLGSDYTEYNEKFKGRVTLTSDTSASTAYMELSSLRSEDTAVYYCARSAGSLFAYWGQGTLVTVSSASTKGPSVFPLAPSSKSTSGGTAALGCLVKDYFPEPVTVSWNSGALTSGVHTFPAVLQSSGLYSLSSVVTVPSSSLGTQTYICNVNHKPSNTKVDKKVEPKSCDKTHTCPPCPAPELLGGPSVFLFPPKPKDTLMISRTPEVTCVVVDVSHEDPEVKFNWYVDGVEVHNAKTKPREEQYNSTYRVVSVLTVLHQDWLNGKEYKCKVSNKALPAPIEKTISKAKGQPREPQVYTLPPSRDELTKNQVSLTCLVKGFYPSDIAVEWESNGQPENNYKTTPPVLDSDGSFFLYSKLTVDKSRWQQGNVFSCSVMHEALHNHYTQKSLSLSPGK

SEQ ID NO: 100 - protein, 214 aa, synthetic construct; identical to SEQ ID NO: 98
  CHAIN 1..214: note = F4-18-H2L1 light chain

SEQ ID NO: 101 - protein, 447 aa, synthetic construct; identical to SEQ ID NO: 99
  CHAIN 1..447: note = F4-18-H2L2 heavy chain

SEQ ID NO: 102 - protein, 214 aa, synthetic construct
  CHAIN 1..214: note = F4-18-H2L2 light chain
DIQMTQSPSSLSASVGDRVTITCRASQDIGITLNWLQQKPGKAPKRLIYATSSLDSGVPSRFSGSRSGTDYTLTISSLQPEDFATYYCLQYASSPYTFGGGTKVEIKRTVAAPSVFIFPPSDEQLKSGTASVVCLLNNFYPREAKVQWKVDNALQSGNSQESVTEQDSKDSTYSLSSTLTLSKADYEKHKVYACEVTHQGLSSPVTKSFNRGEC

SEQ ID NO: 103 - protein, 447 aa, synthetic construct; identical to SEQ ID NO: 99
  CHAIN 1..447: note = F4-18-H2L3 heavy chain

SEQ ID NO: 104 - protein, 214 aa, synthetic construct
  CHAIN 1..214: note = F4-18-H2L3 light chain
DIQLTQSPSSLSASVGDRVTITCRASQDIGITLNWLQQKPGKAIKRLIYATSSLDSGVPSRFSGSRSGSDYTLTISSLQPEDFATYYCLQYASSPYTFGGGTKVEIKRTVAAPSVFIFPPSDEQLKSGTASVVCLLNNFYPREAKVQWKVDNALQSGNSQESVTEQDSKDSTYSLSSTLTLSKADYEKHKVYACEVTHQGLSSPVTKSFNRGEC

SEQ ID NO: 105 - protein, 447 aa, synthetic construct
  CHAIN 1..447: note = F4-18-H4L3 heavy chain
EVQLVQSGAEVVKPGASVKMSCKTSGYTFTSYGINWVRQRPGQGLEWIGYIYLGSDYTEYNEKFKGRVTLTSDTSASTAYMELSSLRSEDTAVYYCARSGGSLFAYWGQGTLVTVSSASTKGPSVFPLAPSSKSTSGGTAALGCLVKDYFPEPVTVSWNSGALTSGVHTFPAVLQSSGLYSLSSVVTVPSSSLGTQTYICNVNHKPSNTKVDKKVEPKSCDKTHTCPPCPAPELLGGPSVFLFPPKPKDTLMISRTPEVTCVVVDVSHEDPEVKFNWYVDGVEVHNAKTKPREEQYNSTYRVVSVLTVLHQDWLNGKEYKCKVSNKALPAPIEKTISKAKGQPREPQVYTLPPSRDELTKNQVSLTCLVKGFYPSDIAVEWESNGQPENNYKTTPPVLDSDGSFFLYSKLTVDKSRWQQGNVFSCSVMHEALHNHYTQKSLSLSPGK

SEQ ID NO: 106 - protein, 214 aa, synthetic construct; identical to SEQ ID NO: 104
  CHAIN 1..214: note = F4-18-H4L3 light chain

SEQ ID NO: 107 - protein, 447 aa, synthetic construct; identical to SEQ ID NO: 97
  CHAIN 1..447: note = F4-18-H1L4 heavy chain

SEQ ID NO: 108 - protein, 214 aa, synthetic construct
  CHAIN 1..214: note = F4-18-H1L4 light chain
DIQLTQSPSSLSASVGDRVTITCRASQDIGITLNWLQQEPGGAIKRLIYATSSLDSGVPKRFSGSRSGSDYTLTISSLQPEDFATYYCLQYASSPYTFGGGTKVEIKRTVAAPSVFIFPPSDEQLKSGTASVVCLLNNFYPREAKVQWKVDNALQSGNSQESVTEQDSKDSTYSLSSTLTLSKADYEKHKVYACEVTHQGLSSPVTKSFNRGEC

SEQ ID NO: 109 - protein, 447 aa, synthetic construct; identical to SEQ ID NO: 99
  CHAIN 1..447: note = F4-18-H2L4 heavy chain

SEQ ID NO: 110 - protein, 214 aa, synthetic construct; identical to SEQ ID NO: 108
  CHAIN 1..214: note = F4-18-H2L4 light chain

SEQ ID NO: 111 - protein, 447 aa, synthetic construct; identical to SEQ ID NO: 105
  CHAIN 1..447: note = F4-18-H4L4 heavy chain

SEQ ID NO: 112 - protein, 214 aa, synthetic construct; identical to SEQ ID NO: 108
  CHAIN 1..214: note = F4-18-H4L4 light chain

SEQ ID NO: 113 - protein, 14 aa, synthetic construct
  REGION 1..14: note = huM6VH5/ huM6VH6/ huM6VH7-HCDR3
YGEDTSGGYYAVDY

SEQ ID NO: 114 - protein, 8 aa, synthetic construct
  CHAIN 1..8: note = huF4-18VH4-HCDR3
SGGSLFAY

SEQ ID NO: 115 - protein, 8 aa, synthetic construct
  CHAIN 1..8: note = huF4-18VH5-HCDR3
SAGSLFGY

SEQ ID NO: 116 - protein, 5 aa, synthetic construct
  REGION 1..5: note = Zalutumumab-HCDR1
TYGMH

SEQ ID NO: 117 - protein, 17 aa, synthetic construct
  REGION 1..17: note = Zalutumumab-HCDR2
VIWDDGSYKYYGDSVKG

SEQ ID NO: 118 - protein, 16 aa, synthetic construct
  REGION 1..16: note = Zalutumumab-HCDR3
DGITMVRGVMKDYFDY

SEQ ID NO: 119 - protein, 11 aa, synthetic construct
  REGION 1..11: note = Zalutumumab-LCDR1
RASQDISSALV

SEQ ID NO: 120 - protein, 7 aa, synthetic construct
  REGION 1..7: note = Zalutumumab-LCDR2
DASSLES

SEQ ID NO: 121 - protein, 9 aa, synthetic construct
  REGION 1..9: note = Zalutumumab-LCDR3
QQFNSYPLT

SEQ ID NO: 122 - protein, 125 aa, synthetic construct [sequence omitted]

SEQ ID NO: 123 - protein, 107 aa, synthetic construct [sequence omitted]

SEQ ID NO: 124 - protein, 455 aa, synthetic construct
  CHAIN 1..455: note = Zalutumumab heavy chain
QVQLVESGGGVVQPGRSLRLSCAASGFTFSTYGMHWVRQAPGKGLEWVAVIWDDGSYKYYGDSVKGRFTISRDNSKNTLYLQMNSLRAEDTAVYYCARDGITMVRGVMKDYFDYWGQGTLVTVSSASTKGPSVFPLAPSSKSTSGGTAALGCLVKDYFPEPVTVSWNSGALTSGVHTFPAVLQSSGLYSLSSVVTVPSSSLGTQTYICNVNHKPSNTKVDKRVEPKSCDKTHTCPPCPAPELLGGPSVFLFPPKPKDTLMISRTPEVTCVVVDVSHEDPEVKFNWYVDGVEVHNAKTKPREEQYNSTYRVVSVLTVLHQDWLNGKEYKCKVSNKALPAPIEKTISKAKGQPREPQVYTLPPSREEMTKNQVSLTCLVKGFYPSDIAVEWESNGQPENNYKTTPPVLDSDGSFFLYSKLTVDKSRWQQGNVFSCSVMHEALHNHYTQKSLSLSPGK

SEQ ID NO: 125 - protein, 214 aa, synthetic construct
  CHAIN 1..214: note = Zalutumumab light chain
AIQLTQSPSSLSASVGDRVTITCRASQDISSALVWYQQKPGKAPKLLIYDASSLESGVPSRFSGSESGTDFTLTISSLQPEDFATYYCQQFNSYPLTFGGGTKVEIKRTVAAPSVFIFPPSDEQLKSGTASVVCLLNNFYPREAKVQWKVDNALQSGNSQESVTEQDSKDSTYSLSSTLTLSKADYEKHKVYACEVTHQGLSSPVTKSFNRGEC

SEQ ID NO: 126 - protein, 5 aa, synthetic construct
  REGION 1..5: note = ZalH1-HCDR1
SYGMH

SEQ ID NO: 127 - protein, 17 aa, synthetic construct
  REGION 1..17: note = ZalH2-HCDR2
VIWEDGSYKYYGDSVKG

SEQ ID NO: 128 - protein, 16 aa, synthetic construct
  REGION 1..16: note = ZalH3-HCDR3
DGLTMVRGVMKDYFDY

SEQ ID NO: 129 - protein, 16 aa, synthetic construct
  REGION 1..16: note = ZalH4-HCDR3
DGVTMVRGVMKDYFDY

SEQ ID NO: 130 - protein, 16 aa, synthetic construct
  REGION 1..16: note = ZalH5-HCDR3
DGATMVRGVMKDYFDY

SEQ ID NO: 131 - protein, 16 aa, synthetic construct
  REGION 1..16: note = ZalH6-HCDR3
DGITVVRGVMKDYFDY

SEQ ID NO: 132 - protein, 17 aa, synthetic construct
  REGION 1..17: note = ZalH12-HCDR2
VIWDDGSNKYYGDSVKG

SEQ ID NO: 133 - protein, 5 aa, synthetic construct
  REGION 1..5: note = ZalH13-HCDR1
SYAMH

SEQ ID NO: 134 - protein, 17 aa, synthetic construct
  REGION 1..17: note = ZalH14-HCDR2
VIWYDGSNKYYADSVKG

SEQ ID NO: 135 - protein, 125 aa, synthetic construct
  REGION 1..125: note = ZalVH1
QVQLVESGGGVVQPGRSLRLSCAASGFTFSSYGMHWVRQAPGKGLEWVAVIWDDGSYKYYGDSVKGRFTISRDNSKNTLYLQMNSLRAEDTAVYYCARDGITMVRGVMKDYFDYWGQGTLVTVSS

SEQ ID NO: 136 - protein, 125 aa, synthetic construct
  REGION 1..125: note = ZalVH2
QVQLVESGGGVVQPGRSLRLSCAASGFTFSTYGMHWVRQAPGKGLEWVAVIWEDGSYKYYGDSVKGRFTISRDNSKNTLYLQMNSLRAEDTAVYYCARDGITMVRGVMKDYFDYWGQGTLVTVSS

SEQ ID NO: 137 - protein, 125 aa, synthetic construct
  REGION 1..125: note = ZalVH3
QVQLVESGGGVVQPGRSLRLSCAASGFTFSTYGMHWVRQAPGKGLEWVAVIWDDGSYKYYGDSVKGRFTISRDNSKNTLYLQMNSLRAEDTAVYYCARDGLTMVRGVMKDYFDYWGQGTLVTVSS

SEQ ID NO: 138 - protein, 125 aa, synthetic construct
  REGION 1..125: note = ZalVH4
QVQLVESGGGVVQPGRSLRLSCAASGFTFSTYGMHWVRQAPGKGLEWVAVIWDDGSYKYYGDSVKGRFTISRDNSKNTLYLQMNSLRAEDTAVYYCARDGVTMVRGVMKDYFDYWGQGTLVTVSS

SEQ ID NO: 139 - protein, 125 aa, synthetic construct
  REGION 1..125: note = ZalVH5
QVQLVESGGGVVQPGRSLRLSCAASGFTFSTYGMHWVRQAPGKGLEWVAVIWDDGSYKYYGDSVKGRFTISRDNSKNTLYLQMNSLRAEDTAVYYCARDGATMVRGVMKDYFDYWGQGTLVTVSS

SEQ ID NO: 140 - protein, 125 aa, synthetic construct
  REGION 1..125: note = ZalVH6
QVQLVESGGGVVQPGRSLRLSCAASGFTFSTYGMHWVRQAPGKGLEWVAVIWDDGSYKYYGDSVKGRFTISRDNSKNTLYLQMNSLRAEDTAVYYCARDGITVVRGVMKDYFDYWGQGTLVTVSS

SEQ ID NO: 141 - protein, 125 aa, synthetic construct
  REGION 1..125: note = ZalVH7
QVQLVESGGGVVQPGRSLRLSCAASGFTFSSYGMHWVRQAPGKGLEWVAVIWEDGSYKYYGDSVKGRFTISRDNSKNTLYLQMNSLRAEDTAVYYCARDGITMVRGVMKDYFDYWGQGTLVTVSS

SEQ ID NO: 142 - protein, 125 aa, synthetic construct
  REGION 1..125: note = ZalVH8
QVQLVESGGGVVQPGRSLRLSCAASGFTFSSYGMHWVRQAPGKGLEWVAVIWDDGSYKYYGDSVKGRFTISRDNSKNTLYLQMNSLRAEDTAVYYCARDGLTMVRGVMKDYFDYWGQGTLVTVSS

SEQ ID NO: 143 - protein, 125 aa, synthetic construct
  REGION 1..125: note = ZalVH9
QVQLVESGGGVVQPGRSLRLSCAASGFTFSSYGMHWVRQAPGKGLEWVAVIWDDGSYKYYGDSVKGRFTISRDNSKNTLYLQMNSLRAEDTAVYYCARDGVTMVRGVMKDYFDYWGQGTLVTVSS

SEQ ID NO: 144 - protein, 125 aa, synthetic construct
  REGION 1..125: note = ZalVH10
QVQLVESGGGVVQPGRSLRLSCAASGFTFSSYGMHWVRQAPGKGLEWVAVIWDDGSYKYYGDSVKGRFTISRDNSKNTLYLQMNSLRAEDTAVYYCARDGATMVRGVMKDYFDYWGQGTLVTVSS

SEQ ID NO: 145 - protein, 125 aa, synthetic construct
  REGION 1..125: note = ZalVH11
QVQLVESGGGVVQPGRSLRLSCAASGFTFSSYGMHWVRQAPGKGLEWVAVIWDDGSYKYYGDSVKGRFTISRDNSKNTLYLQMNSLRAEDTAVYYCARDGITVVRGVMKDYFDYWGQGTLVTVSS

SEQ ID NO: 146 - protein, 125 aa, synthetic construct
  REGION 1..125: note = ZalVH12
QVQLVESGGGVVQPGRSLRLSCAASGFTFSTYGMHWVRQAPGKGLEWVAVIWDDGSNKYYGDSVKGRFTISRDNSKNTLYLQMNSLRAEDTAVYYCARDGITMVRGVMKDYFDYWGQGTLVTVSS

SEQ ID NO: 147 - protein, 125 aa, synthetic construct
  REGION 1..125: note = ZalVH13
QVQLVESGGGVVQPGRSLRLSCAASGFTFSSYAMHWVRQAPGKGLEWVAVIWDDGSYKYYGDSVKGRFTISRDNSKNTLYLQMNSLRAEDTAVYYCARDGITMVRGVMKDYFDYWGQGTLVTVSS

SEQ ID NO: 148 - protein, 125 aa, synthetic construct
  REGION 1..125: note = ZalVH14
QVQLVESGGGVVQPGRSLRLSCAASGFTFSTYGMHWVRQAPGKGLEWVAVIWYDGSNKYYADSVKGRFTISRDNSKNTLYLQMNSLRAEDTAVYYCARDGITMVRGVMKDYFDYWGQGTLVTVSS

SEQ ID NO: 149 - protein, 107 aa, synthetic construct
  REGION 1..107: note = ZalVL1
DIQLTQSPSSLSASVGDRVTITCRASQDISSALVWYQQKPGKAPKLLIYDASSLESGVPSRFSGSESGTDFTLTISSLQPEDFATYYCQQFNSYPLTFGGGTKVEIK

SEQ ID NO: 150 - protein, 455 aa, synthetic construct
  CHAIN 1..455: note = ZalH1 Heavy chain
QVQLVESGGGVVQPGRSLRLSCAASGFTFSSYGMHWVRQAPGKGLEWVAVIWDDGSYKYYGDSVKGRFTISRDNSKNTLYLQMNSLRAEDTAVYYCARDGITMVRGVMKDYFDYWGQGTLVTVSSASTKGPSVFPLAPSSKSTSGGTAALGCLVKDYFPEPVTVSWNSGALTSGVHTFPAVLQSSGLYSLSSVVTVPSSSLGTQTYICNVNHKPSNTKVDKKVEPKSCDKTHTCPPCPAPELLGGPSVFLFPPKPKDTLMISRTPEVTCVVVDVSHEDPEVKFNWYVDGVEVHNAKTKPREEQYNSTYRVVSVLTVLHQDWLNGKEYKCKVSNKALPAPIEKTISKAKGQPREPQVYTLPPSRDELTKNQVSLTCLVKGFYPSDIAVEWESNGQPENNYKTTPPVLDSDGSFFLYSKLTVDKSRWQQGNVFSCSVMHEALHNHYTQKSLSLSPGK

SEQ ID NO: 151 - protein, 455 aa, synthetic construct
  CHAIN 1..455: note = ZalH2 heavy chian
QVQLVESGGGVVQPGRSLRLSCAASGFTFSTYGMHWVRQAPGKGLEWVAVIWEDGSYKYYGDSVKGRFTISRDNSKNTLYLQMNSLRAEDTAVYYCARDGITMVRGVMKDYFDYWGQGTLVTVSSASTKGPSVFPLAPSSKSTSGGTAALGCLVKDYFPEPVTVSWNSGALTSGVHTFPAVLQSSGLYSLSSVVTVPSSSLGTQTYICNVNHKPSNTKVDKKVEPKSCDKTHTCPPCPAPELLGGPSVFLFPPKPKDTLMISRTPEVTCVVVDVSHEDPEVKFNWYVDGVEVHNAKTKPREEQYNSTYRVVSVLTVLHQDWLNGKEYKCKVSNKALPAPIEKTISKAKGQPREPQVYTLPPSRDELTKNQVSLTCLVKGFYPSDIAVEWESNGQPENNYKTTPPVLDSDGSFFLYSKLTVDKSRWQQGNVFSCSVMHEALHNHYTQKSLSLSPGK

SEQ ID NO: 152 - protein, 455 aa, synthetic construct
  CHAIN 1..455: note = ZalH3 heavy chain
QVQLVESGGGVVQPGRSLRLSCAASGFTFSTYGMHWVRQAPGKGLEWVAVIWDDGSYKYYGDSVKGRFTISRDNSKNTLYLQMNSLRAEDTAVYYCARDGLTMVRGVMKDYFDYWGQGTLVTVSSASTKGPSVFPLAPSSKSTSGGTAALGCLVKDYFPEPVTVSWNSGALTSGVHTFPAVLQSSGLYSLSSVVTVPSSSLGTQTYICNVNHKPSNTKVDKKVEPKSCDKTHTCPPCPAPELLGGPSVFLFPPKPKDTLMISRTPEVTCVVVDVSHEDPEVKFNWYVDGVEVHNAKTKPREEQYNSTYRVVSVLTVLHQDWLNGKEYKCKVSNKALPAPIEKTISKAKGQPREPQVYTLPPSRDELTKNQVSLTCLVKGFYPSDIAVEWESNGQPENNYKTTPPVLDSDGSFFLYSKLTVDKSRWQQGNVFSCSVMHEALHNHYTQKSLSLSPGK

SEQ ID NO: 153 - protein, 455 aa, synthetic construct
  CHAIN 1..455: note = ZalH4 heavy chain
QVQLVESGGGVVQPGRSLRLSCAASGFTFSTYGMHWVRQAPGKGLEWVAVIWDDGSYKYYGDSVKGRFTISRDNSKNTLYLQMNSLRAEDTAVYYCARDGVTMVRGVMKDYFDYWGQGTLVTVSSASTKGPSVFPLAPSSKSTSGGTAALGCLVKDYFPEPVTVSWNSGALTSGVHTFPAVLQSSGLYSLSSVVTVPSSSLGTQTYICNVNHKPSNTKVDKKVEPKSCDKTHTCPPCPAPELLGGPSVFLFPPKPKDTLMISRTPEVTCVVVDVSHEDPEVKFNWYVDGVEVHNAKTKPREEQYNSTYRVVSVLTVLHQDWLNGKEYKCKVSNKALPAPIEKTISKAKGQPREPQVYTLPPSRDELTKNQVSLTCLVKGFYPSDIAVEWESNGQPENNYKTTPPVLDSDGSFFLYSKLTVDKSRWQQGNVFSCSVMHEALHNHYTQKSLSLSPGK

SEQ ID NO: 154 - protein, 455 aa, synthetic construct
  CHAIN 1..455: note = ZalH5 heavy chain
QVQLVESGGGVVQPGRSLRLSCAASGFTFSTYGMHWVRQAPGKGLEWVAVIWDDGSYKYYGDSVKGRFTISRDNSKNTLYLQMNSLRAEDTAVYYCARDGATMVRGVMKDYFDYWGQGTLVTVSSASTKGPSVFPLAPSSKSTSGGTAALGCLVKDYFPEPVTVSWNSGALTSGVHTFPAVLQSSGLYSLSSVVTVPSSSLGTQTYICNVNHKPSNTKVDKKVEPKSCDKTHTCPPCPAPELLGGPSVFLFPPKPKDTLMISRTPEVTCVVVDVSHEDPEVKFNWYVDGVEVHNAKTKPREEQYNSTYRVVSVLTVLHQDWLNGKEYKCKVSNKALPAPIEKTISKAKGQPREPQVYTLPPSRDELTKNQVSLTCLVKGFYPSDIAVEWESNGQPENNYKTTPPVLDSDGSFFLYSKLTVDKSRWQQGNVFSCSVMHEALHNHYTQKSLSLSPGK

SEQ ID NO: 155 - protein, 455 aa, synthetic construct
  CHAIN 1..455: note = ZalH6 heavy chain
QVQLVESGGGVVQPGRSLRLSCAASGFTFSTYGMHWVRQAPGKGLEWVAVIWDDGSYKYYGDSVKGRFTISRDNSKNTLYLQMNSLRAEDTAVYYCARDGITVVRGVMKDYFDYWGQGTLVTVSSASTKGPSVFPLAPSSKSTSGGTAALGCLVKDYFPEPVTVSWNSGALTSGVHTFPAVLQSSGLYSLSSVVTVPSSSLGTQTYICNVNHKPSNTKVDKKVEPKSCDKTHTCPPCPAPELLGGPSVFLFPPKPKDTLMISRTPEVTCVVVDVSHEDPEVKFNWYVDGVEVHNAKTKPREEQYNSTYRVVSVLTVLHQDWLNGKEYKCKVSNKALPAPIEKTISKAKGQPREPQVYTLPPSRDELTKNQVSLTCLVKGFYPSDIAVEWESNGQPENNYKTTPPVLDSDGSFFLYSKLTVDKSRWQQGNVFSCSVMHEALHNHYTQKSLSLSPGK

SEQ ID NO: 156 - protein, 455 aa, synthetic construct
  CHAIN 1..455: note = ZalH7 heavy chain
QVQLVESGGGVVQPGRSLRLSCAASGFTFSSYGMHWVRQAPGKGLEWVAVIWEDGSYKYYGDSVKGRFTISRDNSKNTLYLQMNSLRAEDTAVYYCARDGITMVRGVMKDYFDYWGQGTLVTVSSASTKGPSVFPLAPSSKSTSGGTAALGCLVKDYFPEPVTVSWNSGALTSGVHTFPAVLQSSGLYSLSSVVTVPSSSLGTQTYICNVNHKPSNTKVDKKVEPKSCDKTHTCPPCPAPELLGGPSVFLFPPKPKDTLMISRTPEVTCVVVDVSHEDPEVKFNWYVDGVEVHNAKTKPREEQYNSTYRVVSVLTVLHQDWLNGKEYKCKVSNKALPAPIEKTISKAKGQPREPQVYTLPPSRDELTKNQVSLTCLVKGFYPSDIAVEWESNGQPENNYKTTPPVLDSDGSFFLYSKLTVDKSRWQQGNVFSCSVMHEALHNHYTQKSLSLSPGK

SEQ ID NO: 157 - protein, 455 aa, synthetic construct
  CHAIN 1..455: note = ZalH8 heavy chain
QVQLVESGGGVVQPGRSLRLSCAASGFTFSSYGMHWVRQAPGKGLEWVAVIWDDGSYKYYGDSVKGRFTISRDNSKNTLYLQMNSLRAEDTAVYYCARDGLTMVRGVMKDYFDYWGQGTLVTVSSASTKGPSVFPLAPSSKSTSGGTAALGCLVKDYFPEPVTVSWNSGALTSGVHTFPAVLQSSGLYSLSSVVTVPSSSLGTQTYICNVNHKPSNTKVDKKVEPKSCDKTHTCPPCPAPELLGGPSVFLFPPKPKDTLMISRTPEVTCVVVDVSHEDPEVKFNWYVDGVEVHNAKTKPREEQYNSTYRVVSVLTVLHQDWLNGKEYKCKVSNKALPAPIEKTISKAKGQPREPQVYTLPPSRDELTKNQVSLTCLVKGFYPSDIAVEWESNGQPENNYKTTPPVLDSDGSFFLYSKLTVDKSRWQQGNVFSCSVMHEALHNHYTQKSLSLSPGK

SEQ ID NO: 158 - protein, 455 aa, synthetic construct
  CHAIN 1..455: note = ZalH9 heavy chain
QVQLVESGGGVVQPGRSLRLSCAASGFTFSSYGMHWVRQAPGKGLEWVAVIWDDGSYKYYGDSVKGRFTISRDNSKNTLYLQMNSLRAEDTAVYYCARDGVTMVRGVMKDYFDYWGQGTLVTVSSASTKGPSVFPLAPSSKSTSGGTAALGCLVKDYFPEPVTVSWNSGALTSGVHTFPAVLQSSGLYSLSSVVTVPSSSLGTQTYICNVNHKPSNTKVDKKVEPKSCDKTHTCPPCPAPELLGGPSVFLFPPKPKDTLMISRTPEVTCVVVDVSHEDPEVKFNWYVDGVEVHNAKTKPREEQYNSTYRVVSVLTVLHQDWLNGKEYKCKVSNKALPAPIEKTISKAKGQPREPQVYTLPPSRDELTKNQVSLTCLVKGFYPSDIAVEWESNGQPENNYKTTPPVLDSDGSFFLYSKLTVDKSRWQQGNVFSCSVMHEALHNHYTQKSLSLSPGK

SEQ ID NO: 159 - protein, 455 aa, synthetic construct
  CHAIN 1..455: note = ZalH10 heavy chain
QVQLVESGGGVVQPGRSLRLSCAASGFTFSSYGMHWVRQAPGKGLEWVAVIWDDGSYKYYGDSVKGRFTISRDNSKNTLYLQMNSLRAEDTAVYYCARDGATMVRGVMKDYFDYWGQGTLVTVSSASTKGPSVFPLAPSSKSTSGGTAALGCLVKDYFPEPVTVSWNSGALTSGVHTFPAVLQSSGLYSLSSVVTVPSSSLGTQTYICNVNHKPSNTKVDKKVEPKSCDKTHTCPPCPAPELLGGPSVFLFPPKPKDTLMISRTPEVTCVVVDVSHEDPEVKFNWYVDGVEVHNAKTKPREEQYNSTYRVVSVLTVLHQDWLNGKEYKCKVSNKALPAPIEKTISKAKGQPREPQVYTLPPSRDELTKNQVSLTCLVKGFYPSDIAVEWESNGQPENNYKTTPPVLDSDGSFFLYSKLTVDKSRWQQGNVFSCSVMHEALHNHYTQKSLSLSPGK

SEQ ID NO: 160 - protein, 455 aa, synthetic construct
  CHAIN 1..455: note = ZalH11 heavy chain
QVQLVESGGGVVQPGRSLRLSCAASGFTFSSYGMHWVRQAPGKGLEWVAVIWDDGSYKYYGDSVKGRFTISRDNSKNTLYLQMNSLRAEDTAVYYCARDGITVVRGVMKDYFDYWGQGTLVTVSSASTKGPSVFPLAPSSKSTSGGTAALGCLVKDYFPEPVTVSWNSGALTSGVHTFPAVLQSSGLYSLSSVVTVPSSSLGTQTYICNVNHKPSNTKVDKKVEPKSCDKTHTCPPCPAPELLGGPSVFLFPPKPKDTLMISRTPEVTCVVVDVSHEDPEVKFNWYVDGVEVHNAKTKPREEQYNSTYRVVSVLTVLHQDWLNGKEYKCKVSNKALPAPIEKTISKAKGQPREPQVYTLPPSRDELTKNQVSLTCLVKGFYPSDIAVEWESNGQPENNYKTTPPVLDSDGSFFLYSKLTVDKSRWQQGNVFSCSVMHEALHNHYTQKSLSLSPGK

SEQ ID NO: 161 - protein, 455 aa, synthetic construct
  CHAIN 1..455: note = ZalH12 heavy chain
QVQLVESGGGVVQPGRSLRLSCAASGFTFSTYGMHWVRQAPGKGLEWVAVIWDDGSNKYYGDSVKGRFTISRDNSKNTLYLQMNSLRAEDTAVYYCARDGITMVRGVMKDYFDYWGQGTLVTVSSASTKGPSVFPLAPSSKSTSGGTAALGCLVKDYFPEPVTVSWNSGALTSGVHTFPAVLQSSGLYSLSSVVTVPSSSLGTQTYICNVNHKPSNTKVDKKVEPKSCDKTHTCPPCPAPELLGGPSVFLFPPKPKDTLMISRTPEVTCVVVDVSHEDPEVKFNWYVDGVEVHNAKTKPREEQYNSTYRVVSVLTVLHQDWLNGKEYKCKVSNKALPAPIEKTISKAKGQPREPQVYTLPPSRDELTKNQVSLTCLVKGFYPSDIAVEWESNGQPENNYKTTPPVLDSDGSFFLYSKLTVDKSRWQQGNVFSCSVMHEALHNHYTQKSLSLSPGK

SEQ ID NO: 162 - protein, 455 aa, synthetic construct
  CHAIN 1..455: note = ZalH13 heavy chain
QVQLVESGGGVVQPGRSLRLSCAASGFTFSSYAMHWVRQAPGKGLEWVAVIWDDGSYKYYGDSVKGRFTISRDNSKNTLYLQMNSLRAEDTAVYYCARDGITMVRGVMKDYFDYWGQGTLVTVSSASTKGPSVFPLAPSSKSTSGGTAALGCLVKDYFPEPVTVSWNSGALTSGVHTFPAVLQSSGLYSLSSVVTVPSSSLGTQTYICNVNHKPSNTKVDKKVEPKSCDKTHTCPPCPAPELLGGPSVFLFPPKPKDTLMISRTPEVTCVVVDVSHEDPEVKFNWYVDGVEVHNAKTKPREEQYNSTYRVVSVLTVLHQDWLNGKEYKCKVSNKALPAPIEKTISKAKGQPREPQVYTLPPSRDELTKNQVSLTCLVKGFYPSDIAVEWESNGQPENNYKTTPPVLDSDGSFFLYSKLTVDKSRWQQGNVFSCSVMHEALHNHYTQKSLSLSPGK

SEQ ID NO: 163 - protein, 455 aa, synthetic construct
  CHAIN 1..455: note = ZalH14 heavy chain
QVQLVESGGGVVQPGRSLRLSCAASGFTFSTYGMHWVRQAPGKGLEWVAVIWYDGSNKYYADSVKGRFTISRDNSKNTLYLQMNSLRAEDTAVYYCARDGITMVRGVMKDYFDYWGQGTLVTVSSASTKGPSVFPLAPSSKSTSGGTAALGCLVKDYFPEPVTVSWNSGALTSGVHTFPAVLQSSGLYSLSSVVTVPSSSLGTQTYICNVNHKPSNTKVDKKVEPKSCDKTHTCPPCPAPELLGGPSVFLFPPKPKDTLMISRTPEVTCVVVDVSHEDPEVKFNWYVDGVEVHNAKTKPREEQYNSTYRVVSVLTVLHQDWLNGKEYKCKVSNKALPAPIEKTISKAKGQPREPQVYTLPPSRDELTKNQVSLTCLVKGFYPSDIAVEWESNGQPENNYKTTPPVLDSDGSFFLYSKLTVDKSRWQQGNVFSCSVMHEALHNHYTQKSLSLSPGK

SEQ ID NO: 164 - protein, 214 aa, synthetic construct
  CHAIN 1..214: note = light chain
DIQLTQSPSSLSASVGDRVTITCRASQDISSALVWYQQKPGKAPKLLIYDASSLESGVPSRFSGSESGTDFTLTISSLQPEDFATYYCQQFNSYPLTFGGGTKVEIKRTVAAPSVFIFPPSDEQLKSGTASVVCLLNNFYPREAKVQWKVDNALQSGNSQESVTEQDSKDSTYSLSSTLTLSKADYEKHKVYACEVTHQGLSSPVTKSFNRGEC

SEQ ID NO: 165 - protein, 98 aa, synthetic construct
  REGION 1..98: note = Titin
GIPPKIECLPIDISIDEGKVLTVASAFTGEPTPEVTWSTGGRKIHSQEQGRFHIENTDDSTTLTIKDVQKQDGGLYTLTLRNEFGSDSATVNIHIRSI

SEQ ID NO: 166 - protein, 97 aa, synthetic construct
  REGION 1..97: note = Obscurin
SGAPRFLTRPKASVVSVGKDATLSCQIVGNPFPQVSWEKDKQPVTAGVRFRLAQDGDLYRLKILDLQLSDSGQYVCRARNAHGEAFACLGLQVDAEA

SEQ ID NO: 167 - protein, 98 aa, synthetic construct
  REGION 1..98: note = CH1
ASTKGPSVFPLAPSSKSTSGGTAALGCLVKDYFPEPVTVSWNSGALTSGVHTFPAVLQSSGLYSLSSVVTVPSSSLGTQTYICNVNHKPSNTKVDKKV

SEQ ID NO: 168 - protein, 5 aa, synthetic construct
  REGION 1..5: note = linker
GGGGS

SEQ ID NO: 169 - protein, 232 aa, synthetic construct
  REGION 1..232: note = Fc(knob)
EPKSCDKTHTCPPCPAPELLGGPSVFLFPPKPKDTLMISRTPEVTCVVVDVSHEDPEVKFNWYVDGVEVHNAKTKPREEQYNSTYRVVSVLTVLHQDWLNGKEYKCKVSNKALPAPIEKTISKAKGQPREPQVYTLPPCRDELTKNQVSLWCLVKGFYPSDIAVEWESNGQPENNYKTTPPVLDSDGSFFLYSKLTVDKSRWQQGNVFSCSVMHEALHNHYTQKSLSLSPGK

SEQ ID NO: 170 - protein, 227 aa, synthetic construct
  REGION 1..227: note = Fc(hole)
DKTHTCPPCPAPELLGGPSVFLFPPKPKDTLMISRTPEVTCVVVDVSHEDPEVKFNWYVDGVEVHNAKTKPREEQYNSTYRVVSVLTVLHQDWLNGKEYKCKVSNKALPAPIEKTISKAKGQPREPQVCTLPPSRDELTKNQVSLSCAVKGFYPSDIAVEWESNGQPENNYKTTPPVLDSDGSFFLVSKLTVDKSRWQQGNVFSCSVMHEALHNHYTQKSLSLSPGK

SEQ ID NO: 171 - protein, 451 aa, synthetic construct
  CHAIN 1..451: note = M4H1L1-ZalH' chain1
EVQLVQSGAEVKKPGASVKVSCKASGYTFTTYGVPWVRQAPGQGLEWMGDIYPRSGNTYYNEKFKGRVTMTADKSTDTVYMELSSLRSEDTAVYYCAREDYDNYPYALDYWGQGTTVTVSSASTKGPSVFPLAPSSKSTSGGTAALGCLVKDYFPEPVTVSWNSGALTSGVHTFPAVLQSSGLYSLSSVVTVPSSSLGTQTYICNVNHKPSNTKVDKKVEPKSCDKTHTCPPCPAPELLGGPSVFLFPPKPKDTLMISRTPEVTCVVVDVSHEDPEVKFNWYVDGVEVHNAKTKPREEQYNSTYRVVSVLTVLHQDWLNGKEYKCKVSNKALPAPIEKTISKAKGQPREPQVYTLPPCRDELTKNQVSLWCLVKGFYPSDIAVEWESNGQPENNYKTTPPVLDSDGSFFLYSKLTVDKSRWQQGNVFSCSVMHEALHNHYTQKSLSLSPGK

SEQ ID NO: 172 - protein, 455 aa, synthetic construct
  CHAIN 1..455: note = M4H1L1-ZalH'chain 3
QVQLVESGGGVVQPGRSLRLSCAASGFTFSTYGMHWVRQAPGKGLEWVAVIWDDGSYKYYGDSVKGRFTISRDNSKNTLYLQMNSLRAEDTAVYYCARDGITMVRGVMKDYFDYWGQGTLVTVSSGGGGSGIPPKIECLPIDISIDEGKVLTVASAFTGEPTPEVTWSTGGRKIHSQEQGRFHIENTDDSTTLTIKDVQKQDGGLYTLTLRNEFGSDSATVNIHIRSIDKTHTCPPCPAPELLGGPSVFLFPPKPKDTLMISRTPEVTCVVVDVSHEDPEVKFNWYVDGVEVHNAKTKPREEQYNSTYRVVSVLTVLHQDWLNGKEYKCKVSNKALPAPIEKTISKAKGQPREPQVCTLPPSRDELTKNQVSLSCAVKGFYPSDIAVEWESNGQPENNYKTTPPVLDSDGSFFLVSKLTVDKSRWQQGNVFSCSVMHEALHNHYTQKSLSLSPGK

SEQ ID NO: 173 - protein, 209 aa, synthetic construct
  CHAIN 1..209: note = M4H1L1-ZalH'chain4
DIQLTQSPSSLSASVGDRVTITCRASQDISSALVWYQQKPGKAPKLLIYDASSLESGVPSRFSGSESGTDFTLTISSLQPEDFATYYCQQFNSYPLTFGGGTKVEIKGGGGSSGAPRFLTRPKASVVSVGKDATLSCQIVGNPFPQVSWEKDKQPVTAGVRFRLAQDGDLYRLKILDLQLSDSGQYVCRARNAHGEAFACLGLQVDAEA

SEQ ID NO: 174 - protein, 455 aa, synthetic construct
  CHAIN 1..455: note = M4H1L1-ZalH4 chain3
QVQLVESGGGVVQPGRSLRLSCAASGFTFSTYGMHWVRQAPGKGLEWVAVIWDDGSYKYYGDSVKGRFTISRDNSKNTLYLQMNSLRAEDTAVYYCARDGVTMVRGVMKDYFDYWGQGTLVTVSSGGGGSGIPPKIECLPIDISIDEGKVLTVASAFTGEPTPEVTWSTGGRKIHSQEQGRFHIENTDDSTTLTIKDVQKQDGGLYTLTLRNEFGSDSATVNIHIRSIDKTHTCPPCPAPELLGGPSVFLFPPKPKDTLMISRTPEVTCVVVDVSHEDPEVKFNWYVDGVEVHNAKTKPREEQYNSTYRVVSVLTVLHQDWLNGKEYKCKVSNKALPAPIEKTISKAKGQPREPQVCTLPPSRDELTKNQVSLSCAVKGFYPSDIAVEWESNGQPENNYKTTPPVLDSDGSFFLVSKLTVDKSRWQQGNVFSCSVMHEALHNHYTQKSLSLSPGK

SEQ ID NO: 175 - protein, 455 aa, synthetic construct
  CHAIN 1..455: note = M4H1L1-ZalH8 chain3
QVQLVESGGGVVQPGRSLRLSCAASGFTFSSYGMHWVRQAPGKGLEWVAVIWDDGSYKYYGDSVKGRFTISRDNSKNTLYLQMNSLRAEDTAVYYCARDGLTMVRGVMKDYFDYWGQGTLVTVSSGGGGSGIPPKIECLPIDISIDEGKVLTVASAFTGEPTPEVTWSTGGRKIHSQEQGRFHIENTDDSTTLTIKDVQKQDGGLYTLTLRNEFGSDSATVNIHIRSIDKTHTCPPCPAPELLGGPSVFLFPPKPKDTLMISRTPEVTCVVVDVSHEDPEVKFNWYVDGVEVHNAKTKPREEQYNSTYRVVSVLTVLHQDWLNGKEYKCKVSNKALPAPIEKTISKAKGQPREPQVCTLPPSRDELTKNQVSLSCAVKGFYPSDIAVEWESNGQPENNYKTTPPVLDSDGSFFLVSKLTVDKSRWQQGNVFSCSVMHEALHNHYTQKSLSLSPGK

SEQ ID NO: 176 - protein, 455 aa, synthetic construct
  CHAIN 1..455: note = M4H1L1-ZalH10 chain 3
QVQLVESGGGVVQPGRSLRLSCAASGFTFSSYGMHWVRQAPGKGLEWVAVIWDDGSYKYYGDSVKGRFTISRDNSKNTLYLQMNSLRAEDTAVYYCARDGATMVRGVMKDYFDYWGQGTLVTVSSGGGGSGIPPKIECLPIDISIDEGKVLTVASAFTGEPTPEVTWSTGGRKIHSQEQGRFHIENTDDSTTLTIKDVQKQDGGLYTLTLRNEFGSDSATVNIHIRSIDKTHTCPPCPAPELLGGPSVFLFPPKPKDTLMISRTPEVTCVVVDVSHEDPEVKFNWYVDGVEVHNAKTKPREEQYNSTYRVVSVLTVLHQDWLNGKEYKCKVSNKALPAPIEKTISKAKGQPREPQVCTLPPSRDELTKNQVSLSCAVKGFYPSDIAVEWESNGQPENNYKTTPPVLDSDGSFFLVSKLTVDKSRWQQGNVFSCSVMHEALHNHYTQKSLSLSPGK

SEQ ID NO: 177 - protein, 455 aa, synthetic construct
  CHAIN 1..455: note = M4H1L1-ZalH13 chain3
QVQLVESGGGVVQPGRSLRLSCAASGFTFSSYAMHWVRQAPGKGLEWVAVIWDDGSYKYYGDSVKGRFTISRDNSKNTLYLQMNSLRAEDTAVYYCARDGITMVRGVMKDYFDYWGQGTLVTVSSGGGGSGIPPKIECLPIDISIDEGKVLTVASAFTGEPTPEVTWSTGGRKIHSQEQGRFHIENTDDSTTLTIKDVQKQDGGLYTLTLRNEFGSDSATVNIHIRSIDKTHTCPPCPAPELLGGPSVFLFPPKPKDTLMISRTPEVTCVVVDVSHEDPEVKFNWYVDGVEVHNAKTKPREEQYNSTYRVVSVLTVLHQDWLNGKEYKCKVSNKALPAPIEKTISKAKGQPREPQVCTLPPSRDELTKNQVSLSCAVKGFYPSDIAVEWESNGQPENNYKTTPPVLDSDGSFFLVSKLTVDKSRWQQGNVFSCSVMHEALHNHYTQKSLSLSPGK

SEQ ID NO: 178 - protein, 451 aa, synthetic construct
  CHAIN 1..451: note = M4H1L1-ZalH4-LALA chain1
EVQLVQSGAEVKKPGASVKVSCKASGYTFTTYGVPWVRQAPGQGLEWMGDIYPRSGNTYYNEKFKGRVTMTADKSTDTVYMELSSLRSEDTAVYYCAREDYDNYPYALDYWGQGTTVTVSSASTKGPSVFPLAPSSKSTSGGTAALGCLVKDYFPEPVTVSWNSGALTSGVHTFPAVLQSSGLYSLSSVVTVPSSSLGTQTYICNVNHKPSNTKVDKKVEPKSCDKTHTCPPCPAPEAAGGPSVFLFPPKPKDTLMISRTPEVTCVVVDVSHEDPEVKFNWYVDGVEVHNAKTKPREEQYNSTYRVVSVLTVLHQDWLNGKEYKCKVSNKALPAPIEKTISKAKGQPREPQVYTLPPCRDELTKNQVSLWCLVKGFYPSDIAVEWESNGQPENNYKTTPPVLDSDGSFFLYSKLTVDKSRWQQGNVFSCSVMHEALHNHYTQKSLSLSPGK

SEQ ID NO: 179 - protein, 455 aa, synthetic construct
  CHAIN 1..455: note = M4H1L1-ZalH4-LALA chain3
QVQLVESGGGVVQPGRSLRLSCAASGFTFSTYGMHWVRQAPGKGLEWVAVIWDDGSYKYYGDSVKGRFTISRDNSKNTLYLQMNSLRAEDTAVYYCARDGVTMVRGVMKDYFDYWGQGTLVTVSSGGGGSGIPPKIECLPIDISIDEGKVLTVASAFTGEPTPEVTWSTGGRKIHSQEQGRFHIENTDDSTTLTIKDVQKQDGGLYTLTLRNEFGSDSATVNIHIRSIDKTHTCPPCPAPEAAGGPSVFLFPPKPKDTLMISRTPEVTCVVVDVSHEDPEVKFNWYVDGVEVHNAKTKPREEQYNSTYRVVSVLTVLHQDWLNGKEYKCKVSNKALPAPIEKTISKAKGQPREPQVCTLPPSRDELTKNQVSLSCAVKGFYPSDIAVEWESNGQPENNYKTTPPVLDSDGSFFLVSKLTVDKSRWQQGNVFSCSVMHEALHNHYTQKSLSLSPGK

SEQ ID NO: 180 - protein, 4 aa, synthetic construct
  REGION 1..4: note = linker
GGFG

SEQ ID NO: 181 - protein, 4 aa, synthetic construct
  REGION 1..4: note = linker
GGGG

SEQ ID NO: 182 - protein, 232 aa, synthetic construct
  REGION 1..232: note = Fc(knob)'
EPKSCDKTHTCPPCPAPEAAGGPSVFLFPPKPKDTLMISRTPEVTCVVVDVSHEDPEVKFNWYVDGVEVHNAKTKPREEQYNSTYRVVSVLTVLHQDWLNGKEYKCKVSNKALPAPIEKTISKAKGQPREPQVYTLPPCRDELTKNQVSLWCLVKGFYPSDIAVEWESNGQPENNYKTTPPVLDSDGSFFLYSKLTVDKSRWQQGNVFSCSVMHEALHNHYTQKSLSLSPGK

SEQ ID NO: 183 - protein, 227 aa, synthetic construct
  REGION 1..227: note = Fc(hole)'
DKTHTCPPCPAPEAAGGPSVFLFPPKPKDTLMISRTPEVTCVVVDVSHEDPEVKFNWYVDGVEVHNAKTKPREEQYNSTYRVVSVLTVLHQDWLNGKEYKCKVSNKALPAPIEKTISKAKGQPREPQVCTLPPSRDELTKNQVSLSCAVKGFYPSDIAVEWESNGQPENNYKTTPPVLDSDGSFFLVSKLTVDKSRWQQGNVFSCSVMHEALHNHYTQKSLSLSPGK

SEQ ID NO: 184 - protein, 448 aa, synthetic construct
  CHAIN 1..448: note = IgG1 heavy chain
QVQLVQSGAEVKKPGASVKVSCKASGYTFTNSWIGWFRQAPGQGLEWIGDIYPGGGYTNYNEIFKGKATMTADTSTNTAYMELSSLRSEDTAVYYCSRGIPGYAMDYWGQGTLVTVSSASTKGPSVFPLAPSSKSTSGGTAALGCLVKDYFPEPVTVSWNSGALTSGVHTFPAVLQSSGLYSLSSVVTVPSSSLGTQTYICNVNHKPSNTKVDKKVEPKSCDKTHTCPPCPAPELLGGPSVFLFPPKPKDTLMISRTPEVTCVVVDVSHEDPEVKFNWYVDGVEVHNAKTKPREEQYNSTYRVVSVLTVLHQDWLNGKEYKCKVSNKALPAPIEKTISKAKGQPREPQVYTLPPSRDELTKNQVSLTCLVKGFYPSDIAVEWESNGQPENNYKTTPPVLDSDGSFFLYSKLTVDKSRWQQGNVFSCSVMHEALHNHYTQKSLSLSPGK

SEQ ID NO: 185 - protein, 220 aa, synthetic construct
  CHAIN 1..220: note = IgG1 light chain
DIQMTQSPSSLSASVGDRVTMSCKSSQSLLNSGDQKNYLTWYQQKPGKAPKLLIYWASTGESGVPSRFSGSGSGTDFTFTISSLQPEDIATYYCQNDYSYPWTFGQGTKVEIKRTVAAPSVFIFPPSDEQLKSGTASVVCLLNNFYPREAKVQWKVDNALQSGNSQESVTEQDSKDSTYSLSSTLTLSKADYEKHKVYACEVTHQGLSSPVTKSFNRGEC

SEQ ID NO: 186 - protein, 330 aa, synthetic construct
  source 1..330: note = IgG1 HC-LALA
ASTKGPSVFPLAPSSKSTSGGTAALGCLVKDYFPEPVTVSWNSGALTSGVHTFPAVLQSSGLYSLSSVVTVPSSSLGTQTYICNVNHKPSNTKVDKKVEPKSCDKTHTCPPCPAPEAAGGPSVFLFPPKPKDTLMISRTPEVTCVVVDVSHEDPEVKFNWYVDGVEVHNAKTKPREEQYNSTYRVVSVLTVLHQDWLNGKEYKCKVSNKALPAPIEKTISKAKGQPREPQVYTLPPSRDELTKNQVSLTCLVKGFYPSDIAVEWESNGQPENNYKTTPPVLDSDGSFFLYSKLTVDKSRWQQGNVFSCSVMHEALHNHYTQKSLSLSPGK